European Patent Application EP 4 155 407 A1, published March 29, 2023. Title: A thermostable glucocerebrosidase <l30> FTK-0001WO. Applicant: Teikyo University. The sequence listing filed with the application follows.

SEQUENCE LISTING (24 sequences)

SEQ ID NO: 1 - protein, 521 aa [sequence omitted]

SEQ ID NO: 2 - protein, 503 aa
MAFRGGTMLILTMMALLEIQICSSEINRGNFPNGFVFGTASSAFQYEGAVKEDGRGPSVWDTFSHTFGKIIDFSNADVAVDQYHRYEEDIQLMKDMGMDAYRFSISWSRIFPNGYGQINQAGVDHYNKLINALLAKGIEPYVTLYHWDLPQALENKYSGWLNASIIMDFATYAETCFQKFGDRVKHWITFNEPHTFATQGYDVGLQAPGRCSILLHLFCRAGNSATEPYIVAHNVLLSHATVADIYRKKYKKIQGGSLGVAFDVIWYEPLTNTKEDIDAAQRAQDFQLGWFLDPLMFGDYPSSMRTRVGSRLPKFSQSEAALVKGSLDFVGINHYTTFYAKDNSTNLIGTLLHDSIADSGAVTLPFNGTKAISERASSIWLYIVPQSMRSLMIYIKQKYGNPPVYITENGMDDPNSIFISIKDALKDEKRIRYHTGYLSYLLASIKDGCNVKGYFVWSLLDNWEWSAGYTSRFGLYFVDYKDNLKRYPKQSVEWFKNFLKPTK

SEQ ID NO: 3 - DNA, 1566 bp, Oryza sativa L. cv. Nipponbare
atggggaggataaagagtagtagtgggcgatgcagcacggcgaggctggaggcggtcgccgtcctcgtcgtcgtcttcggcgtcgcgtcgtcgtcgctgcgaggatgcattgcgcagcagagcggaggagggctaaccaggggcagcttccccgaggggttcgtcttcggcaccgcctccgccgcgtaccagtacgagggagctgtgaaggaggacgggagagggcagaccatctgggacacgttcgcgcacacctttggaaagatcaccgacttcagcaatgctgatgttgcagttgatcagtaccaccgtttcgaggaggatatacagctcatggcagacatggggatggatgcgtatcggttctcgatagcatggtcaagaatctacccaaatggtgttggtcaagtcaatcaagctggtatcgaccactacaacaagctgatcgatgcacttctagcaaaaggaattcagccatatgtgacactctaccactgggacctcccccaggcccttgaagacaagtacaagggctggcttgacaggcagatagtggacgatttcgcggcgtacgcggagacgtgcttcagggagttcggggacagggtgaagcactggatcacgctcaacgagccgcacacggtggccatccagggctacgacgcagggctccaggcccccggccgctgctccgtgctgctccacctctactgcaaggccggcaactccggcaccgagccctacgtcgtcgcccaccacttcatcctcgcccacgccgccgccgccagcatctacaggacaaaatacaaggcgacgcagaacgggcagcttgggatagcgttcgacgtgatgtggttcgagccgatgtccaacaccacgatcgacatcgaggcggccaagagagcgcaggagtttcagctaggatggtttgctgatccgttcttcttcggcgactacccggcgacgatgagggcgagggtgggggagaggctgccgaggttcacggcggatgaggccgccgtcgtcaagggggcgctggatttcgtcggcataaaccactacaccacctactacacgaggcacaacaacaccaacatcatcgggacattgctcaacaacaccttggcagacaccggcaccgtcagcctcccattcaagaatgggaagccaattggagatagggcaaattcgatatggctgtacattgtgccccgagggatgaggagcctgatgaactatgtcaaggaaaggtacaacagcccaccagtgtacatcactgaaaacgggatggatgacagcaacaacccgttcatttccatcaaggacgccctcaaggacagcaagaggatcaaataccacaatgactacctcaccaatctggctgcttccatcaaggaggacgggtgcgacgtacgtgggtacttcgcgtggtctctgctggacaactgggagtgggcggccggatactcctcgagattcgggctctacttcgtggactacaaggataacctcaagagataccccaagaactcggtgcagtggttcaaggccctcctgaagacctga

SEQ ID NO: 4 - DNA, 1512 bp, Glycine max (L.) Merr. Enrei
atggcgtttagaggaggcactatgttgatattaacaatgatggcattacttgagattcagatatgctcatcggagataaaccgtggaaactttccaaatggcttcgtatttggcactgcctcttcagcttttcagtatgaaggggcagtgaaagaagacggaaggggaccctctgtgtgggacactttttcacatacttttggcaaaataattgatttcagcaatgctgatgttgcggtggatcagtaccaccgatacgaagaagatatacaactgatgaaggacatgggaatggatgcctatagattttccatttcttggtctcggatttttcccaatggatatggccaaatcaatcaggcaggagttgatcattataataaactcatcaacgcgttactagccaaaggaattgaaccatatgtgactctctatcactgggacctgcctcaagccttggaaaacaagtacagtggatggctaaacgcttcaatcataatggactttgcaacttatgctgagacatgctttcagaaatttggggatagggtgaagcattggatcacattcaatgagccacatacatttgccacccaaggatatgatgttggtctacaagcgcctggtcgatgctccattctccttcacctgttttgtagggcggggaactctgctactgaaccttacattgttgcacacaatgtcctactctctcatgcaacagtagcagatatttataggaaaaaatataagaaaatacagggaggatcactaggggtagcttttgatgtcatttggtatgagccactaacaaataccaaagaagacattgatgcagctcaaagagctcaagattttcagctgggctggtttcttgatcctttgatgtttggggattatccaagctcaatgaggactagagtaggaagcaggctaccgaaattttcgcaatcagaagctgctcttgttaagggttcattagattttgttggaatcaatcattacaccacattttatgcaaaagacaattctactaatttaattggaaccctgctccatgattccattgcagactctggtgccgttacccttccattcaatggtactaaagctatttcggaaagggcaagttctatatggctgtatattgtgccacaaagcatgagaagcttaatgatctatatcaaacaaaagtatggaaaccctcctgtctatattacagaaaatgggatggatgatccaaatagtatatttatctccattaaggatgctctaaaggatgaaaaacggatcagataccacactggctatttatcttacttgttggcttctatcaaagatggttgcaatgtgaaaggttattttgtgtggtcactattggataactgggagtggtcagctggatacacgtctagatttggtctatattttgttgactacaaagacaacctgaagagatatcccaaacaatcagtggaatggttcaagaacttcttgaaacctactaaataa

SEQ ID NO: 5 - protein, 130 aa
GSFPEGFVFGTASAAYQYEGAVKEDGRGQTIWDTFAHTFGKITDFSNADVAVDQYHRFEEDIQLMADMGMDAYRFSIAWSRIYPNGVGQVNQAGIDHYNKLIDALLAKGIQPYVTLYHWDLPQALEDKYK

SEQ ID NO: 6 - protein, 15 aa
QIVDDFAAYAETCFR

SEQ ID NO: 7 - protein, 23 aa
AQEFQLGWFADPFFFGDYPATMR

SEQ ID NO: 8 - protein, 17 aa
GALDFVGINHYTTYYTR

SEQ ID NO: 9 - protein, 11 aa
ANSIWLYIVPR

SEQ ID NO: 10 - protein, 7 aa
SLMNYVK

SEQ ID NO: 11 - protein, 24 aa
YNSPPVYITENGMDDSNNPFISIK

SEQ ID NO: 12 - protein, 54 aa
YHNDYLTNLAASIKEDGCDVRGYFAWSLLDNWEWAAGYSSRFGLYFVDYKDNLK

SEQ ID NO: 13 - protein, 7 aa
NSVQWFK

SEQ ID NO: 14 - DNA, 51 bp, Artificial sequence
  F-primer for amplifying Oryza sativa L. cv. Nipponbare Os3BGlu6 gene sequence
tgattacgccaagctgaaggagatatacatatggcgcagcagagcggagga

SEQ ID NO: 15 - DNA, 32 bp, Artificial sequence
  R-primer for amplifying Oryza sativa L. cv. Nipponbare Os3BGlu6 gene sequence
caggcatgcaagcttcaggtcttcaggagggc

SEQ ID NO: 16 - protein, 66 aa
GNFPNGFVFGTASSAFQYEGAVKEDGRGPSVWDTFSHTFGKIIDFSNADVAVDQYHRYEEDIQLMK

SEQ ID NO: 17 - protein, 7 aa
FSISWSR

SEQ ID NO: 18 - protein, 20 aa
GIEPYVTLYHWDLPQALENK

SEQ ID NO: 19 - protein, 27 aa
AGNSATEPYIVAHNVLLSHATVADIYR

SEQ ID NO: 20 - protein, 53 aa
IQGGSLGVAFDVIWYEPLTNTKEDIDAAQRAQDFQLGWFLDPLMFGDYPSSMR

SEQ ID NO: 21 - protein, 17 aa
GSLDFVGINHYTTFYAK

SEQ ID NO: 22 - protein, 13 aa
FGLYFVDYKDNLK

SEQ ID NO: 23 - DNA, 52 bp, Artificial sequence
  F-primer for amplifying Glycine max (L.) Merr. Enrei beta-glucosidase 40 gene sequence
tgattacgccaagctgaaggagatatacatatgattcagatatgctcatcgg

SEQ ID NO: 24 - DNA, 36 bp, Artificial sequence
  R-primer for amplifying Glycine max (L.) Merr. Enrei beta-glucosidase 40 gene sequence
caggcatgcaagctttatttagtaggtttcaagaag